European Patent Specification EP 3 792 628 B1, published April 24, 2024. Title: METHODS FOR PREDICTING THE USEFULNESS OF NEOANTIGENS FOR IMMUNOTHERAPY. Applicant: BioNTech RNA Pharmaceuticals GmbH et al. The sequence listing filed with the application follows.

SEQUENCE LISTING (2 sequences)

SEQ ID NO: 1 - protein, 15 aa, Artificial Sequence
  Linker sequence
  REPEAT (1)..(3): Portion of sequence repeated a times, wherein a is independently a number selected from 0, 1, 2, 3, 4, 5, 6, 7, 8, 9, 10, 11, 12, 13, 14, 15, 16, 17, 18, 19, or 20
  MISC_FEATURE (1)..(15): a + b + c + d + e are different from 0 and preferably are 2 or more, 3 or more, 4 or more or 5 or more
  REPEAT (4)..(6): Portion of sequence repeated b times, wherein b is independently a number selected from 0, 1, 2, 3, 4, 5, 6, 7, 8, 9, 10, 11, 12, 13, 14, 15, 16, 17, 18, 19, or 20
  REPEAT (7)..(9): Portion of sequence repeated c times, wherein c is independently a number selected from 0, 1, 2, 3, 4, 5, 6, 7, 8, 9, 10, 11, 12, 13, 14, 15, 16, 17, 18, 19, or 20
  REPEAT (10)..(12): Portion of sequence repeated d times, wherein d is independently a number selected from 0, 1, 2, 3, 4, 5, 6, 7, 8, 9, 10, 11, 12, 13, 14, 15, 16, 17, 18, 19, or 20
  REPEAT (13)..(15): Portion of sequence repeated e times, wherein e is independently a number selected from 0, 1, 2, 3, 4, 5, 6, 7, 8, 9, 10, 11, 12, 13, 14, 15, 16, 17, 18, 19, or 20
GGSGSSGGGSSGGSG

SEQ ID NO: 2 - protein, 9 aa, Artificial Sequence
  Linker sequence
GGSGGGGSG